European Patent Application EP 4 256 950 A1, published October 11, 2023. Title: TOLERANCE TO CGMMV IN CUCUMBER. Applicant: VILMORIN & CIE. The sequence listing filed with the application follows.

SEQUENCE LISTING (64 sequences)

SEQ ID NO: 1 - DNA, 71 bp, Cucumis sativus
  polymorphism (36)..(36): polymorphism 1 = A; polymorphism 2 = C
ttctaatcctccttatgaggatcatcattttcagartgctgcttctgggcctccgcgggaaagtattttat

SEQ ID NO: 2 - DNA, 71 bp, Cucumis sativus
  Polymorphism (36)..(36): polymorphism 1 = A; polymorphism 2 = G
gtggtggaccataatgtgggattacagagctcgtcrttcatggagtagagaatctggaaagcggattctat

SEQ ID NO: 3 - DNA, 71 bp, Cucumis sativus
  Polymorphism (36)..(36): polymorphism 1 = A; polymorphism 2 = G
aacaaagccaacgtcgaaacataatgattttactaragaagaactcattgccagtaatgtagatagattta

SEQ ID NO: 4 - DNA, 71 bp, Cucumis sativus
  Polymorphism (36)..(36): polymorphism 1 = A; polymorphism 2 = G
ataaacaccacgtcttatctggaggtatagtttcaraactttttctttctaaattcatagaaatagatgtt

SEQ ID NO: 5 - DNA, 71 bp, Cucumis sativus
  Polymorphism (36)..(36): polymorphism 1 = A; polymorphism 2 = G
tttacagtatgagcattggcatcaagaagagtctcragtgatctcgcctttcggctccgaactctaccagc

SEQ ID NO: 6 - DNA, 71 bp, Cucumis sativus
  Polymorphism (36)..(36): polymorphism 1 = A; polymorphism 2 = G
gaaggctctcgagaaaggtaagccatggattagggrcggattcggatggtgaggaaaatggagctgtgtac

SEQ ID NO: 7 - DNA, 71 bp, Cucumis sativus
  Polymorphism (36)..(36): polymorphism 1 = G; polymorphism 2 = C
aaatgtttgaggtttatcagccgacacaagctcctrgtcatttggactgaggaccaaattatcatgaatcc

SEQ ID NO: 8 - DNA, 71 bp, Cucumis sativus
  Polymorphism (36)..(36): polymorphism 1 = A; polymorphism 2 = G
aaaacatacggccatttagcatctaccacagtaacrcatcgtccatccgctcctatgtgtacatagagcca

SEQ ID NO: 9 - DNA, 71 bp, Cucumis sativus
  Polymorphism (36)..(36): susceptible = A; resistant = G
atgaaagagaccccatgttcaaatgaagatgtctcrtaatggaagagggagttccctcaaccaggcaaaaa

SEQ ID NO: 10 - DNA, 71 bp, Cucumis sativus
  Polymorphism (36)..(36): susceptible = A; resistant = G
tcacgttgtagataagatgctcgacttcgaagatcrccatcaatatctcatcttcatactctgcaccgtag

SEQ ID NO: 11 - DNA, 71 bp, Cucumis sativus
  Polymorphism (36)..(36): susceptible = A; resistant = G
gttgcaggatgttgctatgaaatctatgtgaaagcraccatgcgagaagaagctcgacgacaggcaaagac

SEQ ID NO: 12 - DNA, 71 bp, Cucumis sativus
  Polymorphism (36)..(36): susceptible = A; resistant = C
gtgcaagaatttcttcacccaactttattctcccgrgtagacttggtagtagacgagaagtgcttattctg

SEQ ID NO: 13 - DNA, 71 bp, Cucumis sativus
  Polymorphism (36)..(36): susceptible = A; resistant = G
ccacaaactaactgaactaaacagaaaactcacagracagaactacttgtgcaagaatttcttcacccaac

SEQ ID NO: 14 - DNA, 71 bp, Cucumis sativus
  Polymorphism (36)..(36): susceptible = G; resistant = A
atataataaaactgctcataagaagtagaatattcrtccattctttttaattagtttctctctctagatct

SEQ ID NO: 15 - DNA, 71 bp, Cucumis sativus
  Polymorphism (36)..(36): susceptible = G; resistant = A
gcttaccacagccgatgcattcctcatcaccgtcaraagaattcggtagctacgtttccattcactgttga

SEQ ID NO: 16 - DNA, 71 bp, Cucumis sativus
  Polymorphism (36)..(36): susceptible = A; resistant = G
cgaaacctggttccgagttttatccattcatcgtcrccctcaaattcctctgggagctcgtatcttttgag

SEQ ID NO: 17 - DNA, 71 bp, Cucumis sativus
  polymorphism (36)..(36): susceptible = A; resistant = G
gagagagagagagaagagaaaaaaggttggctatgraagaagagggaaaatggggtcatcttataagtggg

SEQ ID NO: 18 - DNA, 71 bp, Cucumis sativus
  Polymorphism (36)..(36): susceptible = A; resistant = G
atgaccaagccattaatcacattagcaccattctcrgctgctcgatcccgaagatacgcgtccagaacctc

SEQ ID NO: 19 - DNA, 71 bp, Cucumis sativus
  Polymorphism (36)..(36): susceptible = G; resistant = A
gcataggttcatttctgaaggtccagtgggctagaraaaagttgacccactagattggggtggcaacttgt

SEQ ID NO: 20 - DNA, 71 bp, Cucumis sativus
  Polymorphism (36)..(36): susceptible = A; resistant = G
tgtacatggtttcgtgctatggctggacttcgaggrggatgcaatttcgacgcatttgttctctgcccaaa

SEQ ID NO: 21 - DNA, 71 bp, Cucumis sativus
  Polymorphism (36)..(36): susceptible = G; resistant = A
gttttggattgctgagaaggagaatgaaggtttccrccatttgaagggatttgaagaacttccatgagaga

SEQ ID NO: 22 - DNA, 71 bp, Cucumis sativus
  Polymorphism (36)..(36): susceptible = A; resistant = G
gaaagggaaagcgagatttatagaggtaagaaaagraaagaaaaaaaagcaaaatcccgactaatttccgg

SEQ ID NO: 23 - DNA, 71 bp, Cucumis sativus
  Polymorphism (36)..(36): susceptible = G; resistant = A
agattataattattataataacaaaacttggtattragagaatcacaccttggacacttcaaagcttggtg

SEQ ID NO: 24 - DNA, 71 bp, Cucumis sativus
  Polymorphism (36)..(36): susceptible = C; resistant = A
agtaacatctttagaaactgaaggagtgccctgctrtgttaaacacgtcgtctttcttagtatacagattt

SEQ ID NO: 25 - DNA, 71 bp, Cucumis sativus
  Polymorphism (36)..(36): susceptible = A; resistant = C
aagcgtcatcaaaaggctgaactcattctgctgcgrgacattgcataaatcccctgagcacgacctatcaa

SEQ ID NO: 26 - DNA, 71 bp, Cucumis sativus
  Polymorphism (36)..(36): susceptible = A; resistant = G
aatcgtatccatttcttccaaactcttcgcctgtargatatggtccagtaaccaaatttaccacctccttg

SEQ ID NO: 27 - DNA, 71 bp, Cucumis sativus
  Polymorphism (36)..(36): susceptible = A; resistant = G
tgggtcgatgtttcttgcgtaggatttggttgctgrgtagaacttacgccaaatgacagcagaattaaaca

SEQ ID NO: 28 - DNA, 71 bp, Cucumis sativus
  Polymorphism (36)..(36): susceptible = A; resistant = G
gaatgcaaaatgaacgtgaccccggcgagaaccaaragtgttccaaccactcgagaacggagaccatgctg

SEQ ID NO: 29 - DNA, 71 bp, Cucumis sativus
  Polymorphism (36)..(36): susceptible = G; resistant = A
gatggaaagccattccattttagttcagagaatgaratttctccttcttctatgattgtccaaaagtgtac

SEQ ID NO: 30 - DNA, 71 bp, Cucumis sativus
  Polymorphism (36)..(36): susceptible = G; resistant = A
tcaggatggaagggtatcattttacgctctcctcgraaacttgtgtgaagctattctctatttttacactc

SEQ ID NO: 31 - DNA, 71 bp, Cucumis sativus
  Polymorphism (36)..(36): susceptible = A; resistant = C
gaaactgaagttgcacataaatttatacactggtgrgtcactgcttccacatcagtttccaaatatacttc

SEQ ID NO: 32 - DNA, 71 bp, Cucumis sativus
  Polymorphism (36)..(36): susceptible = A; resistant = G
ctcggttttgggaagtgtaacactttaacagcttcraagcagtattcagtacacagtaacaaaacgaaata

SEQ ID NO: 33 - DNA, 71 bp, Cucumis sativus
  Polymorphism (36)..(36): susceptible = A; resistant = C
ttcggcgccctttagcttccatgatttagagataargagtattagaagcgagaagagaaagctgagtgttg

SEQ ID NO: 34 - DNA, 71 bp, Cucumis sativus
  Polymorphism (36)..(36): susceptible = G; resistant = A
atgttgatatacccgtccttatcagagtcgagatcrtccatgacagatcgaagctcttctaaggggatggc

SEQ ID NO: 35 - DNA, 71 bp, Cucumis sativus
  Polymorphism (36)..(36): susceptible = G; resistant = A
aactcaggcttagcatcaaacaaacaaacaagcaargcaaggtgcaatacggggatcgataatcaagtaaa

SEQ ID NO: 36 - DNA, 71 bp, Cucumis sativus
  Polymorphism (36)..(36): polymorphism 1 = A; polymorphism 2 = G
gagctcaaccttttgatttagctgcttagctcttcrttgcactgttgttagttttgttatagctgtttgtg

SEQ ID NO: 37 - DNA, 71 bp, Cucumis sativus
  Polymorphism (36)..(36): polymorphism 1 = G; polymorphism 2 = A
gtgggtatgaagctgtagttactaaatattaatgartcattaagtgagaattagcgaagattcagggtttt

SEQ ID NO: 38 - DNA, 71 bp, Cucumis sativus
  Polymorphism (36)..(36): polymorphism 1 = A; polymorphism 2 = G
aaatacaactaagaactttattatgtattaaaaatrtgtcctccgtcgccggcggtagcaatctttaattg

SEQ ID NO: 39 - DNA, 71 bp, Cucumis sativus
  Polymorphism (36)..(36): polymorphism 1 = A; polymorphism 2 = G
tccccaattcaactgatggagaaatcatcatgaaartctaccacttgttttctttggtgcaaaatcttggc

SEQ ID NO: 40 - DNA, 71 bp, Cucumis sativus
  Polymorphism (36)..(36): susceptible = G; resistant = A
gttttagtgttgattattaatgtgttgttgttgatrgggattctgtggttaacccacaaatccatttgtaa

SEQ ID NO: 41 - DNA, 71 bp, Cucumis sativus
  Polymorphism (36)..(36): susceptible = C; resistant = A
attgctgaaaaaagtccaaccttgacctttccgggrggggcttgtccgactgtttgttttggtgggtacct

SEQ ID NO: 42 - DNA, 71 bp, Cucumis sativus
  Polymorphism (36)..(36): susceptible = G; resistant = A
taaaatgagaggtatctataattttatgtataaaargttgactaaactgaagttcatgctaccagggaatt

SEQ ID NO: 43 - DNA, 71 bp, Cucumis sativus
  Polymorphism (36)..(36): susceptible = G; resistant = A
agagaggaaaaagtgggcatccgagcaaaggatctragggttctaggggcgaacattgggtgattcagaag

SEQ ID NO: 44 - DNA, 71 bp, Cucumis sativus
  Polymorphism (36)..(36): susceptible = A; resistant = G
ttccgctggatattttcttctgcagtgaaaaaatcrtcttcttcttgttttccaattccgagtttgggatc

SEQ ID NO: 45 - DNA, 71 bp, Cucumis sativus
  Polymorphism (36)..(36): susceptible = A; resistant = G
tttgataaacccatcytttactcttctccaagttcrtacttcatcctgagtttgagcgagttcaagctcgc

SEQ ID NO: 46 - DNA, 71 bp, Cucumis sativus
  Polymorphism (36)..(36): susceptible = G; resistant = A
gtatcatttttattattattagcttcatcggaggtrttatcaatatcattgcttctggctgggagtttact

SEQ ID NO: 47 - DNA, 71 bp, Cucumis sativus
  Polymorphism (36)..(36): susceptible = A; resistant = G
ttgccaacctcgattgcatctgctaggtcctcagtrgcatctgctctctttgaatagcgttttgcaagttc

SEQ ID NO: 48 - DNA, 71 bp, Cucumis sativus
  Polymorphism (36)..(36): susceptible = G; resistant = A
tggatcatcgtctttggttgttgctggaggtggtcrtattggtgtgatggttgcattgttagggatgtttg

SEQ ID NO: 49 - DNA, 71 bp, Cucumis sativus
  Polymorphism (36)..(36): susceptible = A; resistant = G
ttgttcatagtctttacaacacattagaagaagaarttaaggcaagcttctaagaaagacaaaaggaagct

SEQ ID NO: 50 - DNA, 71 bp, Cucumis sativus
  Polymorphism (36)..(36): susceptible = G; resistant = A
tgactcgtagactgaatgcctccgactgatgtaacracagatcccgaagttggacctacagacatttggtt

SEQ ID NO: 51 - DNA, 71 bp, Cucumis sativus
  Polymorphism (36)..(36): susceptible = A; resistant = G
gatccatgttttcatcttccatttccaacaactccrccacccccaccacctttcaaaacgacaaccatctc

SEQ ID NO: 52 - DNA, 71 bp, Cucumis sativus
  Polymorphism (36)..(36): susceptible = A; resistant = G
tatcttcatgctttctttgataacctagctgacacrgactgcgacgatagctccgatgaaccatgtcagga

SEQ ID NO: 53 - DNA, 71 bp, Cucumis sativus
  Polymorphism (36)..(36): susceptible = C; resistant = A
caagcatgcatctatatttcccatgcggaatcatargaggtgctctttcaaatttgggaattccttgtgcg

SEQ ID NO: 54 - DNA, 71 bp, Cucumis sativus
  Polymorphism (36)..(36): polymorphism 1 = A; polymorphism 2 = G
gtcgttgggggacatgttaaatccatggctgtctaraaggaatttccatatcattgagatctaggtgcaca

SEQ ID NO: 55 - DNA, 71 bp, Cucumis sativus
  Polymorphism (36)..(36): polymorphism 1 = A; polymorphism 2 = G
tcaagatgaggaaaatgaaaacagataaggaatcargatgaggtaaggaactaagaaggagggttcctccc

SEQ ID NO: 56 - DNA, 71 bp, Cucumis sativus
  Polymorphism (36)..(36): polymorphism 1 = A; polymorphism 2 = G
gctctagatagtgttattgatacaatttatttgacraagtcaatgcaaatagttagagaatgacagttaaa

SEQ ID NO: 57 - DNA, 71 bp, Cucumis sativus
  Polymorphism (36)..(36): polymorphism 1 = A; polymorphism 2 = G
tgaagtacctcaaaagccaaatcaagttttaaaaarggtatgctacataggtagagacatttctatatgtc

SEQ ID NO: 58 - DNA, 71 bp, Cucumis sativus
  Polymorphism (36)..(36): susceptible = A; resistant = G
cacagtcgtcacacacaaagttaaagcagcacacargtttatatggttcaaagtatgggggcgtggaagat

SEQ ID NO: 59 - DNA, 71 bp, Cucumis sativus
  Polymorphism (36)..(36): susceptible = A; resistant = G
ttacaggagatgctcacaagacttggtttgaaggartcatgatcaattaaaggggccaccatttttgacca

SEQ ID NO: 60 - DNA, 71 bp, Cucumis sativus
  Polymorphism (36)..(36): susceptible = C; resistant = A
aagaaaacaacttacttcttcaagtgcccaaaagarcctgaatatatggtaagcatgatctttaaacttta

SEQ ID NO: 61 - DNA, 71 bp, Cucumis sativus
  Polymorphism (36)..(36): susceptible = A; resistant = G
acccattgtgtgtccttgtccacatggtgttgcacrccaacttgtcgcctgctaaccacttttggcaagcc

SEQ ID NO: 62 - DNA, 71 bp, Cucumis sativus
  Polymorphism (36)..(36): susceptible = G; resistant = A
catgagaagagaaatttactagggcgtagggccacracgattaacattctaaaacaagcgcggcgacggcg

SEQ ID NO: 63 - DNA, 71 bp, Cucumis sativus
  Polymorphism (36)..(36): susceptible = A; resistant = G
ctctctytcttctctatcaattttacgaagttgcgracgatcaacattccctcgtttgttataatactttc

SEQ ID NO: 64 - DNA, 71 bp, Cucumis sativus
  Polymorphism (36)..(36): susceptible = C; resistant = A
tctttttggattccgggcagccaagcgaatatctgraagaaaagaagtaaaccaataaaaacatattcaat